European Patent Application EP 4 410 980 A1, published August 7, 2024. Title: 細胞濃度の測定方法. Applicant: 武田薬品工業株式会社. The sequence listing filed with the application follows.

SEQUENCE LISTING (9 sequences)

SEQ ID NO: 1 - DNA, 23 bp, synthetic construct
  source 1..23: mol_type = other DNA
tgagttcatatcctttgtaggga

SEQ ID NO: 2 - DNA, 27 bp, synthetic construct
  source 1..27: mol_type = other DNA
ccattactgggtatatacccaaatgag

SEQ ID NO: 3 - DNA, 19 bp, synthetic construct
  source 1..19: mol_type = other DNA
gcgctgcacccactaatgt

SEQ ID NO: 4 - DNA, 30 bp, synthetic construct
  source 1..30: mol_type = other DNA
gccttggctgcgcaggctgctgtggtgcag

SEQ ID NO: 5 - DNA, 27 bp, synthetic construct
  source 1..27: mol_type = other DNA
cgcccatgtattacttcatctgttgcc

SEQ ID NO: 6 - DNA, 21 bp, synthetic construct
  source 1..21: mol_type = other DNA
cacggcgatggcgcccaggaa

SEQ ID NO: 7 - DNA, 15 bp, synthetic construct
  source 1..15: mol_type = other DNA
ttgccccaagtccaa

SEQ ID NO: 8 - DNA, 18 bp, synthetic construct
  source 1..18: mol_type = other DNA
tcgccaagacgagcatca

SEQ ID NO: 9 - DNA, 19 bp, synthetic construct
  source 1..19: mol_type = other DNA
tttgggcgctgaaaaagct